European Patent Application EP 4 711 443 A1, published March 18, 2026. Title: 普利斯特氏菌及其应用. Applicant: 宜宾五粮液股份有限公司. Application CN. The sequence listing filed with the application follows.

SEQUENCE LISTING (3 sequences)

SEQ ID NO: 1 - DNA, 1458 bp, synthetic construct
  source 1..1458: mol_type = other DNA
ggggaatgctacagctagacatgcagtcgagcgaactgattagaagcttgcttctatgacgttagcggcggacgggtgagtaacacgtgggcaacctgcctgtaagactgggataacttcgggaaaccgaagctaataccggataggatcttctccttcatgggagatgattgaaagatggtttcggctatcacttacagatgggcccgcggtgcattagctagttggtgaggtaacggctcaccaaggcaacgatgcatagccgacctgagagggtgatcggccacactgggactgagacacggcccagactcctacgggaggcagcagtagggaatcttccgcaatggacgaaagtctgacggagcaacgccgcgtgagtgatgaaggctttcgggtcgtaaaactctgttgttagggaagaacaagtacgagagtaactgctcgtaccttgacggtacctaaccagaaagccacggctaactacgtgccagcagccgcggtaatacgtaggtggcaagcgttatccggaattattgggcgtaaagcgcgcgcaggcggtttcttaagtctgatgtgaaagcccacggctcaaccgtggagggtcattggaaactggggaacttgagtgcagaagagaaaagcggaattccacgtgtagcggtgaaatgcgtagagatgtggaggaacaccagtggcgaaggcggctttttggtctgtaactgacgctgaggcgcgaaagcgtggggagcaaacaggattagataccctggtagtccacgccgtaaacgatgagtgctaagtgttagagggtttccgccctttagtgctgcagctaacgcattaagcactccgcctggggagtacggtcgcaagactgaaactcaaaggaattgacgggggcccgcacaagcggtggagcatgtggtttaattcgaagcaacgcgaagaaccttaccaggtcttgacatcctctgacaactctagagatagagcgttccccttcgggggacagagtgacaggtggtgcatggttgtcgtcagctcgtgtcgtgagatgttgggttaagtcccgcaacgagcgcaacccttgatcttagttgccagcatttagttgggcactctaaggtgactgccggtgacaaaccggaggaaggtggggatgacgtcaaatcatcatgccccttatgacctgggctacacacgtgctacaatggatggtacaaagggctgcaagaccgcgaggtcaagccaatcccataaaaccattctcagttcggattgtaggctgcaactcgcctacatgaagctggaatcgctagtaatcgcggatcagcatgccgcggtgaatacgttcccgggccttgtacacaccgcccgtcacaccacgagagtttgtaacacccgaagtcggtggagtaaccgtaaggagctagcctacctatagagttccccccg

SEQ ID NO: 2 - DNA, 20 bp, synthetic construct
  source 1..20: mol_type = other DNA
agagtttgatcmtggctcag

SEQ ID NO: 3 - DNA, 19 bp, synthetic construct
  source 1..19: mol_type = other DNA
ggttaccttgttacgactt